European Patent Application EP 4 223 887 A1, published August 9, 2023. Title: Prediction method of COVID-19 aggravation utilizing Protein in exosome. Applicant: International Space Medical Co., Ltd Miyato, Mitsuru Ochiya, Takahiro. The sequence listing filed with the application follows.

SEQUENCE LISTING (36 sequences)

SEQ ID NO: 1 - RNA, 22 nt, Homo sapiens
uggagugugacaaugguguuug

SEQ ID NO: 2 - RNA, 85 nt, Homo sapiens
gcggccggugaugagaacuucucccacucacauucgaguuucccgaccaugagaugacuccacaugcacuaccaucugaggccac

SEQ ID NO: 3 - RNA, 2357 nt, Homo sapiens
gcacucaguacucauggcugaucaagggaagugagcucaucucaccuugacucacagcgaugacagguucaagccccugcaugugggcccguuccucagaggauguuugcaauggggguggggguugccauggugaugcccagucaacagaauggagaaaagagaaauuugguuugaaaugaaauuugagucuugagagagggcugauaugaaggagaaucaaacaagccacaugggagcaucugaaggccuggagauaagggccuguugcauggcugugaaaauuuggccuuuaaaauaacuaggcaugggccagaaaucacagccggcggcugcgaccacccaaggcaggagauccagcgggggacuauggagcucaguggagcugcggccugggagaagcccacccaagagaaccauguaacuagaaaccaucacauucggcuucgugugagggagaagcagguguuucauugcacgcaguuacugagaucugggguuguuuguuauugcagcaaggacccacccuaacacacgagguguuauaugcauuuuacagauugccaagaugguacagacagcagaaguggcaaaacaacacuuaaacucaaaccugcccaacuucaaaguccacgcccuucccugggcuucagacugccgucuuugaugcuaucuuucauugagauguuguuugcauuaaaugggggaucuugcggcacacgguggaccuugcccagcacccacucuuccuagggccagccuuacucuguggggucagccuuugaccgucugggccaugaagguggcugaugaggccccuucgacagccaaguuggggcacaaucuccuccggauguuguuauuccuucacagucucaucgcaggcggggaggaagucagagggcugauuuagaggacagagauacaaacagagugagcagaggauguuuggcugcaguugcuccagaguuucaagggagaaaacacaagcauugcugagcggccauuaggggcuugcacgcucagcugggcacauguccacaccgaggcaucacgugcggucugagcugagcucucaucucuggguuucaggacuuucagcacaguccuggcccuucacguuuagucugggugaucagggauguaaaccagcaauugcaagguggugaagcaccaccguggaagggcaccagccgggcccuggggucacagaagugccccaggaaguguggccguuaagccuggugagaggagagcgagccgggaggacggugagagacaggcaugacggggcggugagugugacugcugcugagcaugucugagacggcaggcagucaccaaaggcuuguaagcagaggcaacacccugacuugugguuuggagagaucauggugacugccgugcagggacggaauggaggcugcuccagugacucuggccgugggcaguggugggcgggugaggggacagaggaaaguggauggaguugcugcccccacaacccugcugagaaagugcccacgggaccuggcggggugugagucacacuugggcugcucugccuggcucugcaccuauuucgugagcuggaagggacagccugagccccgucccuuggauggacaucaaugcaggaguaagggucugucucugaagcucucugagcaacggaagggaaggugcccacugggcucaaugcagagauauuggggcugauguggcaggaggggugggugugcaggcccggcggggaaggagacuuccaaacagacgggcugccccacggggaaucuggcuggggccagucauucucagagucaaaccaucuucauucaacuccgaggcugccccaggccaguagcguccuuccugagagcgcuuccugcgagauuuaugaggcaggggccaggccuggaucguagaaagcuagagaaugccuuggcugcccagggaagucuggaauuucuuccaaaccaagcuuccagacgucccucuggacuccucugucugagaaugggcacuuuaaaggcccaggagagaacucccaugacaccguuuuccaaccucccaucuccccuccccggcagcuccccauuuccggcaucucggcuuggcaggaccccuccaggaccucacuccucugagacgcacugcagaccucacaggugacagcagcguuuugcugacucagaggcaacuaccacgaugacccuccagcccguguccagaccuggggcagcgacuuggacagggggcugcagaagugggucugugagggggaccugacggggggcugcagaagugggucugugaggcggaccugggggggcagcccuggggugggcucacugggg

SEQ ID NO: 4 - RNA, 189 nt, Homo sapiens
caguuuuaugcagaacaucugauuagcaggaucaaacggucaacauuaagcauauguauauuauuuucaaccaucucccugcuccaaaaauccacuuaauauauuguccugggauagaggaaguaccagauauuaaacugauaaaagcagauucuacacuugaucuuagccaaaagaccuagaagggau

SEQ ID NO: 5 - RNA, 3857 nt, Homo sapiens
agcuacauccgucaccugacacggcccuaccaggaacagccgcgcucccgcggauucuggugcugcucgcguccccgcuccccuauuccccuuauuuuauuccuggcuccccucgucgaaagucuuccauucuucaaacuagauuauuuaaaaaugaaaaaggaagaaaggaaagcgaggucaucucauugcucuauccgccaaucaggaggcugaaugucaguuuugaacuaaaagccgcuccgcuccucuucuagauuuggaaaacaagcgaaauuaaacuaaaccgcugcacgccucugacgcgacaucuggacacggcgcggcgcuggcgcugccggagcugucgacccggccuggcgccggacuaggacuauuugccacgacauuucaaaggauuccaagagagaauauugguguccaugcugugaugauuccucagcuccucucaucugaucuccguccuggcccccaugacuuucuuugugguaguuagggugugguaugugccacugaggcccacaccuauugcugcaauuuauagcacugaucugucaucaauaccacuugcugucuuggaugugaagaugauuuuuccugcagggauucccucuacaaaauuaaaaacacugggcauguggaaauaauauucaugcuuuaaauugucuuuucucuucacuacaccagggguccccaaccccuaggccacagacuguggcccuaguguagugaauagaaaagacaauuuaaagcgugaauauuauuuccucaugcccaguguuuuuaauuuuguacuggucuguggcuuguuagaaaccaggcugcacagcagaaggugggcagcagauauugagaaaccacagaaagagagaaguuaaauaauuuuccugucaaagaccacaucaaugaugaagccagaauuugagcucauguacuuaaccacuggacuaccugccugcccugucgaggaacagcuaagugucccuuuugaugagaagaauaagccucauucugauucaacagcagagaucaaagaaaagacuucuguuuucuggccaccagauauauguuaucugugcuuaaagaauugaaaaacacacaucaaaggagaauuuucuuggaaagagaggguucaagcaucacuguuaggugugcuggaauccuuucccgagucaguacugcuuucuagaagaaaaccggggagaucuauuuggaauguaucuaacuccaaagaaaccaucagagguaacaguagagacgggguuucaccauguuggccagacuggucuugaacucucgaccucgugauucgcccgccucggccucccaaagugcugggauuacaggugugagacaccacacccggcggauagagagaauuuugacagucucuccaaugaacgccuucacugauauccaaagcaugaaggacacaccagggaaaaacauagaccuaacacaggacaaauggaauuauuagaaacauuuucuagcagaagaacacuauucuguugccauuugaaucuuugcuucuuucuagguuugacaaugagccuaucauauaagcccaaauguaaacagaaagagguugaaucagucacgauaagcccaauuaugcugugguaacaaacaaccucaaaaucucauuggcuuaaaauauacagaauuauucuuacucauggcacauauccaucuaucaucugcaggggaucugcucacugaagucacuuaggaacuuggacugauggaacggccacuuuuuggucacuauauguauuaaucuguuuuaauccugcugauaaagacccaaaauugggaacaaaaagaaguuuaacuagacuuacaguuccgcauggcugaggaggccucagaaucauggugggaggcgaaaggcacuucuuacaugguggcagcaagagaaaaaugaggaagaagcaaaagcggaaaccucugauaaacccaucagaucuuaugagacuuauuccacuaucaagagaauagcaugggaaagacuggcucccauaauuuaccucccucugggucccucccucaacaugugggaauucugggagaaacaauucaagauaugacacauucauaauuuaaacagaagccuacgaagaacucauaaauuaaaagaagauaaucuuuucacaaggugauggaggcuuuuuauuuugccacaaaaccacuggugacguugccuguggccaccuuggagaagacacuggaggccugggacauggagacugcuuuucugcagaaaccacaucccuuggaguaaugagcuacaccuaccucaauuauucagugcaguacaacacuccagacagggucucacucugucacccaggcuggaguguauuggcaugauuacagcucacugcaaccuugaacucccaggcucaaaccugagcagcugggacuacagaugcaccaccaugcaugguaccagagauauaauaaugagaaacagacaugcucccuccccucauugagguuacagcuuaguguggagacacacagaugccuaacgcacuaugguauggaaggugcuauggacacagugcucaaauccaugaucuacauagguggagaacuucaguagaggaaguggcaggaauuugggaaugaggagcacagugauuaaacuggggccauucauaugagaguuuaagaacucagaccagugacuuagauuggcuucucucacauggcaagaaacauugcugcuagcacuucccgaguucuacguucuacaacauccaccacuggaucuuaacauagacguaagaucaaaugcaauagcaugucaaacaauguguaacuccaguuauacaaacauuacuguaucucauuggggauacgaagcucuacacacuugaagauggugaaggaauauaaaaaucuaugucucacaguccagacuuggaguacaaguaauaagaagaauaaaacuuaaucccuuaaguagauucaccauaaguuagcucagagcaauuccagugcaaguauggucugugauccaguaguaucuuacagacagcaaguugaacauugugggaugcaugagcuauugaggccuuugcagcuuucugcuacauggaggcuagggccagagucaagauuuaugcuuugcagcacacuggucagcuguuuuugcaaaucagauuaaaugauuuuuaaaugaggcugagagcaugggagauacuaauguguguuuccuugugagcuacugcauaaguuaggaaauugaaauacagaaagaugaaaagugauuugcccaagcauauagaucaaagcuguggcagaaccaggacuggaaccuauaucucucuacuaaugguuuuuuuaaaaaaauaaccuuguuucaaaaauauuaaaaagucacaagaaagguaaacauguggauaaacaaaaugaagaaaauaaaaauuauccaguaauaacauauuggcauaugucuuucugguauauuuuccuguguugucaucauuaucaucuccaucaucauuauauccaucauuaucaucaucaucaucaucaucaucaucauuaucaucaccauagugaacauguaaugcuuaccuagugccagaugcugucuaggcauuuuacauguguuacugguaacucauguaauccucauaacaaccuuauaaggugguugcuauuauccccauguuacauaugaagagacagaagcauaaagaaguugcaccgcugguaauuggcugggauuugaacuuaagcagucuaaccuuagaguaaugauuuuaacaacuaugcuauauacauacaaauuuacaaaauaaaacugggcucagacaauaaaaaaaaaaaaaaaaaaaaaaaaa

SEQ ID NO: 6 - RNA, 1689 nt, Homo sapiens
ggguggggccagauaggagaacaaaagcaggcugcccgagcuagcaguggcaacaugcucaggucucuuaccacgcuguggaagcuuuguucuuucgcucuuugcaaugaauccugcugcugcucacucuuuggguccacacugccuuuaugagcuguaacacucacugugaagguccgcagcuucccuccugagccagcgagaccaggaacccaccagaaggaagaaacucagaacacaucccaacaucagaaggaacaaacuccagacgcgccaccuuaagagcuguaacacucaccgcgagggucugcggcuucauucuucaaaguccauucuaaguuguucugucagugaaacucuguuuaaaacauggcuuguaugaaguugucaggaaucggcucugacacuuggaugauucuucagcuggcuauaaaauucuaaaaucagaguaaccguguauugacuuccaacauuccacauuuccaaagguguuuccugugaucucugggauccugauccgcaccacucaacuuuggccuccuaaacuucauccuugaccccaccccaggaccucuugaccagaauuuauccagcacuccagcacggcuugcacguuaucuggaguaaagagaccuucugggauuucaucagccuccuguccaucaagaguucuuccaguuuuugacugacugaauuuucagugaacugugugucuaacugaagcuuugagagagagagagagagaaagaaggaaaaaaagaaaagguuuuacuucacuugaacuuguuaaaaaggaagagacacagauccagcauaguagaaggagaaagaaagcagacaacaguuuggaauggaggcauugagacggaagaguccauuggagauggaauguacacacaaaaauaacaauuuagguccuuugcucaugcaacaucuuguucuaauguccucugcuccaggucacaacauugagcuacaaagugugugcagugacuccagucugcauucaugcuacaagaugauccguuuaguaagacugagcaaggcuuguuaaccucuuggacgugagagauuuccccugagaaaauauauaaaacaagagaaaagaaagaaaaucaaguacgaucacugaaaaccugcuuaguaguagcaacuauuuacuguagcugauuuuugugcaaggucaacacugaacccuuuaaguccaucuuaguucaaaccucaugaccaaccugccuuccccccucccucccuccacugacacgucaaacaaaacuauccucccucccuccacccuccuaccccucccaaauccuuccuccccacugcaaacagacugaugguuucacagcacagauuagcaaaucauaaaacauauccauaaaugcuccaucaaggcuuagcaaugaagcaacaccuagguucccaacugauuauaaacauguuacaacaaaucuuaguaagcugcucugaaagauaaugugagugcauucuuguucaauggcugaaauuaaugucacauuuauaaauaucuagaaauguagaggauacgauuuaauuaaauaaaaugcaguuuuugagggugugauucaugaaacucaagauugagucuguucccuaucuuacauaauaauggauaaaaaggugccaauuauauaucugaagauaaaagucuacuuguucccuguu

SEQ ID NO: 7 - RNA, 22 nt, Homo sapiens
ugagguaguagguuguaugguu

SEQ ID NO: 8 - RNA, 22 nt, Homo sapiens
uagcuuaucagacugauguuga

SEQ ID NO: 9 - RNA, 21 nt, Homo sapiens
uaccacaggguagaaccacgg

SEQ ID NO: 10 - RNA, 2175 nt, Homo sapiens
cggaggaggggagaggagaggaaagugggaggagaggcugcacucuaaacagcccucuugccugagcaaucugacgcagaggcacaugaggaaucagcacggaaccaucgacccacaggguuaaucccaaugucaauaccugcuagaugucagggauccccugggcugcuggcgagccauuugaaaugacccaucuccugccaccuuggccugcuccucugggccaccucucuccaccugcacuugcuuaccgcuggagggcuggggucugccgucaccugccucucaagaaaccugugccuccagcagccaccgggauccacugggacugugacccuccugccaagaagacccaggaaaagccugcuggccacugucgaugagaggcaggcucccaccugcaggguguucacuuuguggcuccuuccaauaagucaagcaagauggaaacauucgagcgaugcaaggcagcgcuacuuggggaaagagacacugguaugccacaucagcgaggaccaccaggaaagacgauuccuuuccaaauuccaagccucaacaaaagcgaccacagcaguccagacuccugucucuaaucccuacuuccccauguggacaaagaguggggcucuuuuggccugagcucaugggguuucacaucagcccagcaggacagaaugcaucccuccugacagccaggcacaggcuggggaccagagagacccagcuggcuccacagggcagggcugacacagagccaggggaggguuguggcggcccacacugcaugucucuacaaggugaaggaacuccuuguguuggcugcugagcugagaggucacagcucugccucacagcacccuggccaaguuuuccaugaaaucauccaaagccaacaggaguuccgggaaccauccaucuggagcugcagcuuccucccuggcuguggggaucuucagaucccuugggccugggauaaguccacucuccacacauguaggggaaacaugccagagggccagcccuuguucccagacacggcccuggccccuagcaagccugcucagacacagggggaugguuacagcagaccuaccuagcuggcuaaugucucccuaguagccaauuaauugcagcauucacugagggacuaggcagucaugcagaggccaagcucuaaagggcacccaccccagccugucccccaacaacccagacacacagacccacagcuacaucccugugcaaaugccauaaucccagcuuggcugcacgaacaugcgcaccucucccauccauggcagcgggcccaaagggcaggcaacaggcagaaagcagcuggacacuagggguaagcugaggaagaccagcccucggccccuuccucucuacacagagugguggggagacaaggaggagcgagggauacugacccgggccugaggaacaccugacccagcagcacagaacagagaugagaaaugggccccauuuccaucccccaaauccuucaagaugaccacugaagcugcaaaaaaucaauuuucugcagcuucuucggaagccaggauuuauuuucugugugugcagagcuauuggcucagcuguuucccaucagcuuccugcaugcuuccaggcagagcacagcccacugccucccucuccuucuuccucccgcaaugcucaaacccacacccaagguagaccccuaggaaaagcagagggucuugacuugggaaaaucaagccacgugucaggaguucaccccuggauaucaccaccucauguuuccagaguccccagucacuugcaaaggaccucacacaugccccggcuaggagacaaggcuaaagccuguggagucagaggacgagagagagagagagagagagagagaaggggcaggacagaagagccgcuggaccccagauucacagggcacaaaugcauucucuaggugguaacaucagagccaccacuucucagugucaguccauauuuacugagugccgacugcccgggacccugugccagagcugcgccccaaccccauccaucccgagcuucaugauaauaacauuauucuuuccaacuuugggcugaucaggguuuauaagggcucccacuucacuuuuuaccaaaagaaaauaucuuuccuuugcaaaaaaaaaaaaaaaa

SEQ ID NO: 11 - protein, 906 aa, Homo sapiens
MPLRLDIKRKLTARSDRVKSVDLHPTEPWMLASLYNGSVCVWNHETQTLVKTFEVCDLPVRAAKFVARKNWVVTGADDMQIRVFNYNTLERVHMFEAHSDYIRCIAVHPTQPFILTSSDDMLIKLWDWDKKWSCSQVFEGHTHYVMQIVINPKDNNQFASASLDRTIKVWQLGSSSPNFTLEGHEKGVNCIDYYSGGDKPYLISGADDRLVKIWDYQNKTCVQTLEGHAQNVSCASFHPELPIIITGSEDGTVRIWHSSTYRLESTLNYGMERVWCVASLRGSNNVALGYDEGSIIVKLGREEPAMSMDANGKIIWAKHSEVQQANLKAMGDAEIKDGERLPLAVKDMGSCEIYPQTIQHNPNGRFVVVCGDGEYIIYTAMALRNKSFGSAQEFAWAHDSSEYAIRESNSIVKIFKNFKEKKSFKPDFGAESIYGGFLLGVRSVNGLAFYDWDNTELIRRIEIQPKHIFWSDSGELVCIATEESFFILKYLSEKVLAAQETHEGVTEDGIEDAFEVLGEIQEIVKTGLWVGDCFIYTSSVNRLNYYVGGEIVTIAHLDRTMYLLGYIPKDNRLYLGDKELNIISYSLLVSVLEYQTAVMRRDFSMADKVLPTIPKEQRTRVAHFLEKQGFKQQALTVSTDPEHRFELALQLGELKIAYQLAVEAESEQKWKQLAELAISKCQFGLAQECLHHAQDYGGLLLLATASGNANMVNKLAEGAERDGKNNVAFMSYFLQGKVDACLELLIRTGRLPEAAFLARTYLPSQVSRVVKLWRENLSKVNQKAAESLADPTEYENLFPGLKEAFVVEEWVKETHADLWPAKQYPLVTPNEERNVMEEGKDFQPSRSTAQQELDGKPASPTPVIVASHTANKEEKSLLELEVDLDNLELEDIDTTDINLDEDILDD

SEQ ID NO: 12 - protein, 189 aa, Homo sapiens [sequence omitted]

SEQ ID NO: 13 - protein, 671 aa, Homo sapiens
MADPAAGPPPSEGEESTVRFARKGALRQKNVHEVKNHKFTARFFKQPTFCSHCTDFIWGFGKQGFQCQVCCFVVHKRCHEFVTFSCPGADKGPASDDPRSKHKFKIHTYSSPTFCDHCGSLLYGLIHQGMKCDTCMMNVHKRCVMNVPSLCGTDHTERRGRIYIQAHIDRDVLIVLVRDAKNLVPMDPNGLSDPYVKLKLIPDPKSESKQKTKTIKCSLNPEWNETFRFQLKESDKDRRLSVEIWDWDLTSRNDFMGSLSFGISELQKASVDGWFKLLSQEEGEYFNVPVPPEGSEANEELRQKFERAKISQGTKVPEEKTTNTVSKFDNNGNRDRMKLTDFNFLMVLGKGSFGKVMLSERKGTDELYAVKILKKDVVIQDDDVECTMVEKRVLALPGKPPFLTQLHSCFQTMDRLYFVMEYVNGGDLMYHIQQVGRFKEPHAVFYAAEIAIGLFFLQSKGIIYRDLKLDNVMLDSEGHIKIADFGMCKENIWDGVTTKTFCGTPDYIAPEIIAYQPYGKSVDWWAFGVLLYEMLAGQAPFEGEDEDELFQSIMEHNVAYPKSMSKEAVAICKGLMTKHPGKRLGCGPEGERDIKEHAFFRYIDWEKLERKEIQPPYKPKARDKRDTSNFDKEFTRQPVELTPTDKLFIMNLDQNEFAGFSYTNPEFVINV

SEQ ID NO: 14 - protein, 193 aa, Homo sapiens
MAAIRKKLVIVGDGACGKTCLLIVFSKDQFPEVYVPTVFENYIADIEVDGKQVELALWDTAGQEDYDRLRPLSYPDTDVILMCFSIDSPDSLENIPEKWTPEVKHFCPNVPIILVGNKKDLRQDEHTRRELAKMKQEPVRSEEGRDMANRISAFGYLECSAKTKEGVREVFEMATRAGLQVRKNKRRRGCPIL

SEQ ID NO: 15 - protein, 269 aa, Homo sapiens [sequence omitted]

SEQ ID NO: 16 - protein, 610 aa, Homo sapiens
MAGIAAKLAKDREAAEGLGSHERAIKYLNQDYEALRNECLEAGTLFQDPSFPAIPSALGFKELGPYSSKTRGIEWKRPTEICADPQFIIGGATRTDICQGALGDCWLLAAIASLTLNEEILARVVPLNQSFQENYAGIFHFQFWQYGEWVEVVVDDRLPTKDGELLFVHSAEGSEFWSALLEKAYAKINGCYEALSGGATTEGFEDFTGGIAEWYELKKPPPNLFKIIQKALQKGSLLGCSIDITSAADSEAITFQKLVKGHAYSVTGAEEVESNGSLQKLIRIRNPWGEVEWTGRWNDNCPSWNTIDPEERERLTRRHEDGEFWMSFSDFLRHYSRLEICNLTPDTLTSDTYKKWKLTKMDGNWRRGSTAGGCRNYPNTFWMNPQYLIKLEEEDEDEEDGESGCTFLVGLIQKHRRRQRKMGEDMHTIGFGIYEVPEELSGQTNIHLSKNFFLTNRARERSDTFINLREVLNRFKLPPGEYILVPSTFEPNKDGDFCIRVFSEKKADYQAVDDEIEANLEEFDISEDDIDDGFRRLFAQLAGEDAEISAFELQTILRRVLAKRQDIKSDGFSIETCKIMVDMLDSDGSGKLGLKEFYILWTKIQKKKKK

SEQ ID NO: 17 - protein, 540 aa, Homo sapiens
MGTTARAALVLTYLAVASAASEGGFTATGQRQLRPEHFQEVGYAAPPSPPLSRSLPMDHPDSSQHGPPFEGQSQVQPPPSQEATPLQQEKLLPAQLPAEKEVGPPLPQEAVPLQKELPSLQHPNEQKEGTPAPFGDQSHPEPESWNAAQHCQQDRSQGGWGHRLDGFPPGRPSPDNLNQICLPNRQHVVYGPWNLPQSSYSHLTRQGETLNFLEIGYSRCCHCRSHTNRLECAKLVWEEAMSRFCEAEFSVKTRPHWCCTRQGEARFSCFQEEAPQPHYQLRACPSHQPDISSGLELPFPPGVPTLDNIKNICHLRRFRSVPRNLPATDPLQRELLALIQLEREFQRCCRQGNNHTCTWKAWEDTLDKYCDREYAVKTHHHLCCRHPPSPTRDECFARRAPYPNYDRDILTIDIGRVTPNLMGHLCGNQRVLTKHKHIPGLIHNMTARCCDLPFPEQACCAEEEKLTFINDLCGPRRNIWRDPALCCYLSPGDEQVNCFNINYLRNVALVSGDTENAKGQGEQGSTGGTNISSTSEPKEE

SEQ ID NO: 18 - protein, 437 aa, Homo sapiens
MSWSLHPRNLILYFYALLFLSSTCVAYVATRDNCCILDERFGSYCPTTCGIADFLSTYQTKVDKDLQSLEDILHQVENKTSEVKQLIKAIQLTYNPDESSKPNMIDAATLKSRKMLEEIMKYEASILTHDSSIRYLQEIYNSNNQKIVNLKEKVAQLEAQCQEPCKDTVQIHDITGKDCQDIANKGAKQSGLYFIKPLKANQQFLVYCEIDGSGNGWTVFQKRLDGSVDFKKNWIQYKEGFGHLSPTGTTEFWLGNEKIHLISTQSAIPYALRVELEDWNGRTSTADYAMFKVGPEADKYRLTYAYFAGGDAGDAFDGFDFGDDPSDKFFTSHNGMQFSTWDNDNDKFEGNCAEQDGSGWWMNKCHAGHLNGVYYQGGTYSKASTPNGYDNGIIWATWKTRWYSMKKTTMKIIPFNRLTIGEGQQHHLGGAKQAGDV

SEQ ID NO: 19 - protein, 255 aa, Homo sapiens
MKALLALPLLLLLSTPPCAPQVSGIRGDALERFCLQQPLDCDDIYAQGYQSDGVYLIYPSGPSVPVPVFCDMTTEGGKWTVFQKRFNGSVSFFRGWNDYKLGFGRADGEYWLGLQNMHLLTLKQKYELRVDLEDFENNTAYAKYADFSISPNAVSAEEDGYTLFVAGFEDGGVGDSLSYHSGQKFSTFDRDQDLFVQNCAALSSGAFWFRSCHFANLNGFYLGGSHLSYANGINWAQWKGFYYSLKRTEMKIRRA

SEQ ID NO: 20 - protein, 179 aa, Homo sapiens
MVQAWYMDDAPGDPRQPHRPDPGRPVGLEQLRRLGVLYWKLDADKYENDPELEKIRRERNYSWMDIITICKDKLPNYEEKIKMFYEEHLHLDDEIRYILDGSGYFDVRDKEDQWIRIFMEKGDMVTLPAGIYHRFTVDEKNYTKAMRLFVGEPVWTAYNRPADHFEARGQYVKFLAQTA

SEQ ID NO: 21 - protein, 194 aa, Homo sapiens
MEEKLKKTKIIFVVGGPGSGKGTQCEKIVQKYGYTHLSTGDLLRSEVSSGSARGKKLSEIMEKGQLVPLETVLDMLRDAMVAKVNTSKGFLIDGYPREVQQGEEFERRIGQPTLLLYVDAGPETMTQRLLKRGETSGRVDDNEETIKKRLETYYKATEPVIAFYEKRGIVRKVNAEGSVDSVFSQVCTHLDALK

SEQ ID NO: 22 - protein, 445 aa, Homo sapiens
MLKKQSAGLVLWGAILFVAWNALLLLFFWTRPAPGRPPSVSALDGDPASLTREVIRLAQDAEVELERQRGLLQQIGDALSSQRGRVPTAAPPAQPRVPVTPAPAVIPILVIACDRSTVRRCLDKLLHYRPSAELFPIIVSQDCGHEETAQAIASYGSAVTHIRQPDLSSIAVPPDHRKFQGYYKIARHYRWALGQVFRQFRFPAAVVVEDDLEVAPDFFEYFRATYPLLKADPSLWCVSAWNDNGKEQMVDASRPELLYRTDFFPGLGWLLLAELWAELEPKWPKAFWDDWMRRPEQRQGRACIRPEISRTMTFGRKGVSHGQFFDQHLKFIKLNQQFVHFTQLDLSYLQREAYDRDFLARVYGAPQLQVEKVRTNDRKELGEVRVQYTGRDSFKAFAKALGVMDDLKSGVPRAGYRGIVTFQFRGRRVHLAPPLTWEGYDPSWN

SEQ ID NO: 23 - protein, 220 aa, Homo sapiens
MSMGLEITGTALAVLGWLGTIVCCALPMWRVSAFIGSNIITSQNIWEGLWMNCVVQSTGQMQCKVYDSLLALPQDLQAARALIVVAILLAAFGLLVALVGAQCTNCVQDDTAKAKITIVAGVLFLLAALLTLVPVSWSANTIIRDFYNPVVPEAQKREMGAGLYVGWAAAALQLLGGALLCCSCPPREKKYTATKVVYSAPRSTGPGASLGTGYDRKDYV

SEQ ID NO: 24 - protein, 224 aa, Homo sapiens
MEKLLCFLVLTSLSHAFGQTDMSRKAFVFPKESDTSYVSLKAPLTKPLKAFTVCLHFYTELSSTRGYSIFSYATKRQDNEILIFWSKDIGYSFTVGGSEILFEVPEVTVAPVHICTSWESASGIVEFWVDGKPRVRKSLKKGYTVGAEASIILGQEQDSFGGNFEGSQSLVGDIGNVNMWDFVLSPDEINTIYLGGPFSPNVLNWRALKYEVQGEVFTKPQLWP

SEQ ID NO: 25 - protein, 453 aa, Homo sapiens
MKLLTRAGSFSRFYSLKVAPKVKATAAPAGAPPQPQDLEFTKLPNGLVIASLENYSPVSRIGLFIKAGSRYEDFSNLGTTHLLRLTSSLTTKGASSFKITRGIEAVGGKLSVTATRENMAYTVECLRGDVDILMEFLLNVTTAPEFRRWEVADLQPQLKIDKAVAFQNPQTHVIENLHAAAYRNALANPLYCPDYRIGKVTSEELHYFVQNHFTSARMALIGLGVSHPVLKQVAEQFLNMRGGLGLSGAKANYRGGEIREQNGDSLVHAAFVAESAVAGSAEANAFSVLQHVLGAGPHVKRGSNTTSHLHQAVAKATQQPFDVSAFNASYSDSGLFGIYTISQATAAGDVIKAAYNQVKTIAQGNLSNTDVQAAKNKLKAGYLMSVESSECFLEEVGSQALVAGSYMPPSTVLQQIDSVANADIINAAKKFVSGQKSMAASGNLGHTPFVDEL

SEQ ID NO: 26 - protein, 644 aa, Homo sapiens
MFSMRIVCLVLSVVGTAWTADSGEGDFLAEGGGVRGPRVVERHQSACKDSDWPFCSDEDWNYKCPSGCRMKGLIDEVNQDFTNRINKLKNSLFEYQKNNKDSHSLTTNIMEILRGDFSSANNRDNTYNRVSEDLRSRIEVLKRKVIEKVQHIQLLQKNVRAQLVDMKRLEVDIDIKIRSCRGSCSRALAREVDLKDYEDQQKQLEQVIAKDLLPSRDRQHLPLIKMKPVPDLVPGNFKSQLQKVPPEWKALTDMPQMRMELERPGGNEITRGGSTSYGTGSETESPRNPSSAGSWNSGSSGPGSTGNRNPGSSGTGGTATWKPGSSGPGSTGSWNSGSSGTGSTGNQNPGSPRPGSTGTWNPGSSERGSAGHWTSESSVSGSTGQWHSESGSFRPDSPGSGNARPNNPDWGTFEEVSGNVSPGTRREYHTEKLVTSKGDKELRTGKEKVTSGSTTTTRRSCSKTVTKTVIGPDGHKEVTKEVVTSEDGSDCPEAMDLGTLSGIGTLDGFRHRHPDEAAFFDTASTGKTFPGFFSPMLGEFVSETESRGSESGIFTNTKESSSHHPGIAEFPSRGKSSSYSKQFTSSTSYNRGDSTFESKSYKMADEAGSEADHEGTHSTKRGHAKSRPVRGIHTSPLGKPSLSP

SEQ ID NO: 27 - protein, 491 aa, Homo sapiens
MKRMVSWSFHKLKTMKHLLLLLLCVFLVKSQGVNDNEEGFFSARGHRPLDKKREEAPSLRPAPPPISGGGYRARPAKAAATQKKVERKAPDAGGCLHADPDLGVLCPTGCQLQEALLQQERPIRNSVDELNNNVEAVSQTSSSSFQYMYLLKDLWQKRQKQVKDNENVVNEYSSELEKHQLYIDETVNSNIPTNLRVLRSILENLRSKIQKLESDVSAQMEYCRTPCTVSCNIPVVSGKECEEIIRKGGETSEMYLIQPDSSVKPYRVYCDMNTENGGWTVIQNRQDGSVDFGRKWDPYKQGFGNVATNTDGKNYCGLPGEYWLGNDKISQLTRMGPTELLIEMEDWKGDKVKAHYGGFTVQNEANKYQISVNKYRGTAGNALMDGASQLMGENRTMTIHNGMFFSTYDRDNDGWLTSDPRKQCSKEDGGGWWYNRCHAANPNGRYYWGGQYTWDMAKHGTDDGVVWMNWKGSWYSMRKMSMKIRPFFPQQ

SEQ ID NO: 28 - protein, 312 aa, Homo sapiens
MAKVFSFILVTTALTMGREISALEDCAQEQMRLRAQVRLLETRVKQQQVKIKQLLQENEVQFLDKGDENTVIDLGSKRQYADCSEIFNDGYKLSGFYKIKPLQSPAEFSVYCDMSDGGGWTVIQRRSDGSENFNRGWKDYENGFGNFVQKHGEYWLGNKNLHFLTTQEDYTLKIDLADFEKNSRYAQYKNFKVGDEKNFYELNIGEYSGTAGDSLAGNFHPEVQWWASHQRMKFSTWDRDHDNYEGNCAEEDQSGWWFNRCHSANLNGVYYSGPYTAKTDNGIVWYTWHGWWYSLKSVVMKIRPNDFIPNVI

SEQ ID NO: 29 - protein, 203 aa, Homo sapiens
  MISC_FEATURE (49)..(49): X=Selenocystein
MCAARLAAAAAAAQSVYAFSARPLAGGEPVSLGSLRGKVLLIENVASLXGTTVRDYTQMNELQRRLGPRGLVVLGFPCNQFGHQENAKNEEILNSLKYVRPGGGFEPNFMLFEKCEVNGAGAHPLFAFLREALPAPSDDATALMTDPKLITWSPVCRNDVAWNFEKFLVGPDGVPLRRYSRRFQTIDIEPDIEALLSQGPSCA

SEQ ID NO: 30 - protein, 433 aa, Homo sapiens
MSGRPRTTSFAESCKPVQQPSAFGSMKVSRDKDGSKVTTVVATPGQGPDRPQEVSYTDTKVIGNGSFGVVYQAKLCDSGELVAIKKVLQDKRFKNRELQIMRKLDHCNIVRLRYFFYSSGEKKDEVYLNLVLDYVPETVYRVARHYSRAKQTLPVIYVKLYMYQLFRSLAYIHSFGICHRDIKPQNLLLDPDTAVLKLCDFGSAKQLVRGEPNVSYICSRYYRAPELIFGATDYTSSIDVWSAGCVLAELLLGQPIFPGDSGVDQLVEIIKVLGTPTREQIREMNPNYTEFKFPQIKAHPWTKDSSGTGHFTSGVRVFRPRTPPEAIALCSRLLEYTPTARLTPLEACAHSFFDELRDPNVKLPNGRDTPALFNFTTQELSSNPPLATILIPPHARIQAAASTPTNATAASDANTGDRGQTNNAASASASNST

SEQ ID NO: 31 - protein, 481 aa, Homo sapiens
MGALARALPSILLALLLTSTPEALGANPGLVARITDKGLQYAAQEGLLALQSELLRITLPDFTGDLRIPHVGRGRYEFHSLNIHSCELLHSALRPVPGQGLSLSISDSSIRVQGRWKVRKSFFKLQGSFDVSVKGISISVNLLLGSESSGRPTVTASSCSSDIADVEVDMSGDLGWLLNLFHNQIESKFQKVLESRICEMIQKSVSSDLQPYLQTLPVTTEIDSFADIDYSLVEAPRATAQMLEVMFKGEIFHRNHRSPVTLLAAVMSLPEEHNKMVYFAISDYVFNTASLVYHEEGYLNFSITDDMIPPDSNIRLTTKSFRPFVPRLARLYPNMNLELQGSVPSAPLLNFSPGNLSVDPYMEIDAFVLLPSSSKEPVFRLSVATNVSATLTFNTSKITGFLKPGKVKVELKESKVGLFNAELLEALLNYYILNTFYPKFNDKLAEGFPLPLLKRVQLYDLGLQIHKDFLFLGANVQYMRV

SEQ ID NO: 32 - protein, 345 aa, Homo sapiens
MSLFGLLLLTSALAGQRQGTQAESNLSSKFQFSSNKEQNGVQDPQHERIITVSTNGSIHSPRFPHTYPRNTVLVWRLVAVEENVWIQLTFDERFGLEDPEDDICKYDFVEVEEPSDGTILGRWCGSGTVPGKQISKGNQIRIRFVSDEYFPSEPGFCIHYNIVMPQFTEAVSPSVLPPSALPLDLLNNAITAFSTLEDLIRYLEPERWQLDLEDLYRPTWQLLGKAFVFGRKSRVVDLNLLTEEVRLYSCTPRNFSVSIREELKRTDTIFWPGCLLVKRCGGNCACCLHNCNECQCVPSKVTKKYHEVLQLRPKTGVRGLHKSLTDVALEHHEECDCVCRGSTGG

SEQ ID NO: 33 - protein, 203 aa, Homo sapiens
MAKAYDHLFKLLLIGDSGVGKTCLIIRFAEDNFNNTYISTIGIDFKIRTVDIEGKKIKLQVWDTAGQERFKTITTAYYRGAMGIILVYDITDEKSFENIQNWMKSIKENASAGVERLLLGNKCDMEAKRKVQKEQADKLAREHGIRFFETSAKSSMNVDEAFSSLARDILLKSGGRRSGNGNKPPSTDLKTCDKKNTNKCSLG

SEQ ID NO: 34 - protein, 184 aa, Homo sapiens
MREYKLVVLGSGGVGKSALTVQFVQGIFVEKYDPTIEDSYRKQVEVDAQQCMLEILDTAGTEQFTAMRDLYMKNGQGFALVYSITAQSTFNDLQDLREQILRVKDTDDVPMILVGNKCDLEDERVVGKEQGQNLARQWNNCAFLESSAKSKINVNEIFYDLVRQINRKTPVPGKARKKSSCQLL

SEQ ID NO: 35 - protein, 630 aa, Homo sapiens
METTPLNSQKQLSACEDGEDCQENGVLQKVVPTPGDKVESGQISNGYSAVPSPGAGDDTRHSIPATTTTLVAELHQGERETWGKKVDFLLSVIGYAVDLGNVWRFPYICYQNGGGAFLLPYTIMAIFGGIPLFYMELALGQYHRNGCISIWRKICPIFKGIGYAICIIAFYIASYYNTIMAWALYYLISSFTDQLPWTSCKNSWNTGNCTNYFSEDNITWTLHSTSPAEEFYTRHVLQIHRSKGLQDLGGISWQLALCIMLIFTVIYFSIWKGVKTSGKVVWVTATFPYIILSVLLVRGATLPGAWRGVLFYLKPNWQKLLETGVWIDAAAQIFFSLGPGFGVLLAFASYNKFNNNCYQDALVTSVVNCMTSFVSGFVIFTVLGYMAEMRNEDVSEVAKDAGPSLLFITYAEAIANMPASTFFAIIFFLMLITLGLDSTFAGLEGVITAVLDEFPHVWAKRRERFVLAVVITCFFGSLVTLTFGGAYVVKLLEEYATGPAVLTVALIEAVAVSWFYGITQFCRDVKEMLGFSPGWFWRICWVAISPLFLLFIICSFLMSPPQLRLFQYNYPYWSIILGYCIGTSSFICIPTYIAYRLIITPGTFKERIIKSITPETPTEIPCGDIRLNAV

SEQ ID NO: 36 - protein, 1012 aa, Homo sapiens
MDALDASKLLDEELYSRQLYVLGSPAMQRIQGARVLVSGLQGLGAEVAKNLVLMGVGSLTLHDPHPTCWSDLAAQFLLSEQDLERSRAEASQELLAQLNRAVQVVVHTGDITEDLLLDFQVVVLTAAKLEEQLKVGTLCHKHGVCFLAADTRGLVGQLFCDFGEDFTVQDPTEAEPLTAAIQHISQGSPGILTLRKGANTHYFRDGDLVTFSGIEGMVELNDCDPRSIHVREDGSLEIGDTTTFSRYLRGGAITEVKRPKTVRHKSLDTALLQPHVVAQSSQEVHHAHCLHQAFCALHKFQHLHGRPPQPWDPVDAETVVGLARDLEPLKRTEEEPLEEPLDEALVRTVALSSAGVLSPMVAMLGAVAAQEVLKAISRKFMPLDQWLYFDALDCLPEDGELLPSPEDCALRGSRYDGQIAVFGAGFQEKLRRQHYLLVGAGAIGCELLKVFALVGLGAGNSGGLTVVDMDHIERSNLSRQFLFRSQDVGRPKAEVAAAAARGLNPDLQVIPLTYPLDPTTEHIYGDNFFSRVDGVAAALDSFQARRYVAARCTHYLKPLLEAGTSGTWGSATVFMPHVTEAYRAPASAAASEDAPYPVCTVRYFPSTAEHTLQWARHEFEELFRLSAETINHHQQAHTSLADMDEPQTLTLLKPVLGVLRVRPQNWQDCVAWALGHWKLCFHYGIKQLLRHFPPNKVLEDGTPFWSGPKQCPQPLEFDTNQDTHLLYVLAAANLYAQMHGLPGSQDWTALRELLKLLPQPDPQQMAPIFASNLELASASAEFGPEQQKELNKALEVWSVGPPLKPLMFEKDDDSNFHVDFVVAAASLRCQNYGIPPVNRAQSKRIVGQIIPAIATTTAAVAGLLGLELYKVVSGPRPRSAFRHSYLHLAENYLIRYMPFAPAIQTFHHLKWTSWDRLKVPAGQPERTLESLLAHLQEQHGLRVRILLHGSALLYAAGWSPEKQAQHLPLRVTELVQQLTGQAPAPGQRVLVLELSCEGDDEDTAFPPLHYEL